European Patent Specification EP 3 957 754 B1, published January 28, 2026. Title: Method for Detecting Chikungunya Vivus. Applicant: Gen-Probe Incorporated Carrick, James M Linnen, Jeffrey M. Application TBA. The sequence listing filed with the application follows.

SEQUENCE LISTING (191 sequences)

SEQ ID NO: 1 - DNA, 152 bp, Chikungunya virus
  misc_feature (1)..(1): n is a, c, g, or t
  misc_feature (67)..(67): n is a, c, g, or t
  misc_feature (144)..(144): n is a, c, g, or t
nacatgcagggtgcctaaagcaaggaaccccaccgtgacgtacgggaaaaaccaagtcatcatgctnctgtatcctgaccacccaacactcctgtcctaccggaatatgggagaagaaccaaactatcaagaagagtgggtgangcataaga

SEQ ID NO: 2 - DNA, 148 bp, Chikungunya virus
  misc_feature (37)..(37): n is a, c, g, or t
  misc_feature (54)..(55): n is a, c, g, or t
  misc_feature (57)..(57): n is a, c, g, or t
  misc_feature (110)..(110): n is a, c, g, or t
tgggagaagaaccaaactatcaagaagagtgggtgangcataagaaggaagtcnngntaaccgtgccgactgaagggctcgaggtcacgtggggcaacaacgagccgtanaagtattggccgcagttatctacaaacggtacagccca

SEQ ID NO: 3 - DNA, 156 bp, Chikungunya virus
  misc_feature (7)..(7): n is a, c, g, or t
  misc_feature (148)..(148): n is a, c, g, or t
taagtangaccttgaatgcgcgcagatacccgtgcacatgaagtccgacgcttcgaagttcacccatgagaaaccggaggggtactacaactggcaccacggagcagtacagtactcaggaggccggttcaccatccctacaggtgcnggcaaacc

SEQ ID NO: 4 - DNA, 84 bp, Chikungunya virus
  misc_feature (82)..(82): n is a, c, g, or t
cggtgcccacactgtgagcgcgtacgaacacgtaacagtgatcccgaacacggtgggagtaccgtataagactctagtcaanag

SEQ ID NO: 5 - DNA, 108 bp, Chikungunya virus
  misc_feature (4)..(4): n is a, c, g, or t
  misc_feature (38)..(38): n is a, c, g, or t
  misc_feature (47)..(47): n is a, c, g, or t
  misc_feature (101)..(101): n is a, c, g, or t
cagnggggatgtgcatgtgtgcacgacgcagatgcatnacaccgtangaactgacaccaggagctaccgtccctttcctgcttagcctaatatgctgcatnagaacag

SEQ ID NO: 6 - DNA, 134 bp, Chikungunya virus
  misc_feature (44)..(44): n is a, c, g, or t
  misc_feature (75)..(75): n is a, c, g, or t
  misc_feature (83)..(83): n is a, c, g, or t
  misc_feature (89)..(89): n is a, c, g, or t
tacctgactacagctgtaaggtcttcaccggcgtctacccattnatgtggggcggcgcctactgcttctgcgacnctgaaaanacgcanttgagcgaagcacatgtggagaagtccgaatcatgcaaaacagaa

SEQ ID NO: 7 - DNA, 88 bp, Chikungunya virus
  misc_feature (4)..(4): n is a, c, g, or t
  misc_feature (10)..(10): n is a, c, g, or t
  misc_feature (82)..(82): n is a, c, g, or t
aaantgggcngatgagcaggtactgaaggctaagaacataggattatgttcaacagacctgacggaaggtagacgaggcaanttgtct

SEQ ID NO: 8 - DNA, 81 bp, Chikungunya virus
  misc_feature (10)..(10): n is a, c, g, or t
  misc_feature (73)..(73): n is a, c, g, or t
  misc_feature (76)..(76): n is a, c, g, or t
gagaaagctngcatctgccgcaggaaaagtcctggacagaaacatctctggaaagatcggggacttacaagcngtnatggc

SEQ ID NO: 9 - DNA, 138 bp, Chikungunya virus
  misc_feature (6)..(6): n is a, c, g, or t
  misc_feature (9)..(9): n is a, c, g, or t
  misc_feature (30)..(30): n is a, c, g, or t
  misc_feature (136)..(136): n is a, c, g, or t
ggcaanctnagcttcacatgccgctgtganacagtggtttcgtgtgagggctacgtcgttaagagaataacgatgagcccaggcctttatggaaaaaccacagggtatgcggtaacccaccacgcagacggattcntg

SEQ ID NO: 10 - DNA, 151 bp, Chikungunya virus
  misc_feature (42)..(42): n is a, c, g, or t
  misc_feature (101)..(101): n is a, c, g, or t
aaaccacagggtatgcggtaacccaccacgcagacggattcntgatgtgcaagactaccgacacggttgacggcgaaagagtgtcattctcggtgtgcacntacgtgccggcgaccatttgtgatcaaatgaccggcatccttgctacaga

SEQ ID NO: 11 - DNA, 146 bp, Chikungunya virus
  misc_feature (53)..(53): n is a, c, g, or t
gcaagactaccgacacggttgacggcgaaagagtgtcattctcggtgtgcacntacgtgccggcgaccatttgtgatcaaatgaccggcatccttgctacagaagtcacgccggaggatgcacagaagctgttggtggggctgaac

SEQ ID NO: 12 - DNA, 97 bp, Chikungunya virus
  misc_feature (40)..(40): n is a, c, g, or t
gaacacactacagaatgtactggcagcagccacgaaaagnaactgcaacgtcacacagatgagggaattacccactttggactcagcagtattcaac

SEQ ID NO: 13 - DNA, 91 bp, Chikungunya virus
  misc_feature (10)..(10): n is a, c, g, or t
  misc_feature (34)..(34): n is a, c, g, or t
  misc_feature (85)..(85): n is a, c, g, or t
aagaacactnacctgctgctgtctatgggcattnaagaagcagaaaacacacacggtctacaagaggcctgatacccagtcaatncagaag

SEQ ID NO: 14 - DNA, 167 bp, Chikungunya virus
  misc_feature (50)..(50): n is a, c, g, or t
  misc_feature (56)..(56): n is a, c, g, or t
  misc_feature (116)..(116): n is a, c, g, or t
acccgaagcagtgcggcttcttcaatatgatgcagatgaaagtcaactanaatcanaacatctgcacccaagtgtaccacaaaagtatctccaggcggtgtacactgcctgtgacngccattgtgtcatcgttgcattacgaaggcaaaatgcgcactacgaatgag

SEQ ID NO: 15 - DNA, 120 bp, Chikungunya virus
  misc_feature (1)..(1): n is a, c, g, or t
  misc_feature (118)..(118): n is a, c, g, or t
nggtaatgtccatggccacctttgcaagctccagatccaacttcgagaagctcagaggacccgtcataactttgtacggcggtcctaaataggtacgcactacagctacctattttgnca

SEQ ID NO: 16 - DNA, 132 bp, Chikungunya virus
  misc_feature (57)..(57): n is a, c, g, or t
gtgcctaaagcaaggaaccccaccgtgacgtacgggaaaaaccaagtcatcatgctnctgtatcctgaccacccaacactcctgtcctaccggaatatgggagaagaaccaaactatcaagaagagtgggtg

SEQ ID NO: 17 - DNA, 127 bp, Chikungunya virus
  misc_feature (26)..(26): n is a, c, g, or t
  misc_feature (43)..(44): n is a, c, g, or t
  misc_feature (46)..(46): n is a, c, g, or t
  misc_feature (99)..(99): n is a, c, g, or t
ccaaactatcaagaagagtgggtgangcataagaaggaagtcnngntaaccgtgccgactgaagggctcgaggtcacgtggggcaacaacgagccgtanaagtattggccgcagttatctacaaacg

SEQ ID NO: 18 - DNA, 136 bp, Chikungunya virus
cttgaatgcgcgcagatacccgtgcacatgaagtccgacgcttcgaagttcacccatgagaaaccggaggggtactacaactggcaccacggagcagtacagtactcaggaggccggttcaccatccctacaggtg

SEQ ID NO: 19 - DNA, 64 bp, Chikungunya virus
actgtgagcgcgtacgaacacgtaacagtgatcccgaacacggtgggagtaccgtataagactc

SEQ ID NO: 20 - DNA, 88 bp, Chikungunya virus
  misc_feature (28)..(28): n is a, c, g, or t
  misc_feature (37)..(37): n is a, c, g, or t
gtgcatgtgtgcacgacgcagatgcatnacaccgtangaactgacaccaggagctaccgtccctttcctgcttagcctaatatgctgc

SEQ ID NO: 21 - DNA, 115 bp, Chikungunya virus
  misc_feature (34)..(34): n is a, c, g, or t
  misc_feature (65)..(65): n is a, c, g, or t
  misc_feature (73)..(73): n is a, c, g, or t
  misc_feature (79)..(79): n is a, c, g, or t
cagctgtaaggtcttcaccggcgtctacccattnatgtggggcggcgcctactgcttctgcgacnctgaaaanacgcanttgagcgaagcacatgtggagaagtccgaatcatgc

SEQ ID NO: 22 - DNA, 68 bp, Chikungunya virus
gatgagcaggtactgaaggctaagaacataggattatgttcaacagacctgacggaaggtagacgagg

SEQ ID NO: 23 - DNA, 62 bp, Chikungunya virus
gcatctgccgcaggaaaagtcctggacagaaacatctctggaaagatcggggacttacaagc

SEQ ID NO: 24 - DNA, 118 bp, Chikungunya virus
  misc_feature (20)..(20): n is a, c, g, or t
gcttcacatgccgctgtganacagtggtttcgtgtgagggctacgtcgttaagagaataacgatgagcccaggcctttatggaaaaaccacagggtatgcggtaacccaccacgcaga

SEQ ID NO: 25 - DNA, 131 bp, Chikungunya virus
  misc_feature (32)..(32): n is a, c, g, or t
  misc_feature (91)..(91): n is a, c, g, or t
gtatgcggtaacccaccacgcagacggattcntgatgtgcaagactaccgacacggttgacggcgaaagagtgtcattctcggtgtgcacntacgtgccggcgaccatttgtgatcaaatgaccggcatcc

SEQ ID NO: 26 - DNA, 124 bp, Chikungunya virus
  misc_feature (42)..(42): n is a, c, g, or t
gacacggttgacggcgaaagagtgtcattctcggtgtgcacntacgtgccggcgaccatttgtgatcaaatgaccggcatccttgctacagaagtcacgccggaggatgcacagaagctgttgg

SEQ ID NO: 27 - DNA, 77 bp, Chikungunya virus
  misc_feature (30)..(30): n is a, c, g, or t
cagaatgtactggcagcagccacgaaaagnaactgcaacgtcacacagatgagggaattacccactttggactcagc

SEQ ID NO: 28 - DNA, 71 bp, Chikungunya virus
  misc_feature (24)..(24): n is a, c, g, or t
acctgctgctgtctatgggcattnaagaagcagaaaacacacacggtctacaagaggcctgatacccagtc

SEQ ID NO: 29 - DNA, 147 bp, Chikungunya virus
  misc_feature (40)..(40): n is a, c, g, or t
  misc_feature (46)..(46): n is a, c, g, or t
  misc_feature (106)..(106): n is a, c, g, or t
gtgcggcttcttcaatatgatgcagatgaaagtcaactanaatcanaacatctgcacccaagtgtaccacaaaagtatctccaggcggtgtacactgcctgtgacngccattgtgtcatcgttgcattacgaaggcaaaatgcgcac

SEQ ID NO: 30 - DNA, 100 bp, Chikungunya virus
catggccacctttgcaagctccagatccaacttcgagaagctcagaggacccgtcataactttgtacggcggtcctaaataggtacgcactacagctacc

SEQ ID NO: 31 - DNA, 44 bp, Chikungunya virus
  misc_feature (9)..(9): n is a, c, g, or t
tcttatgcntcacccactcttcttgatagtttggttcttctccc

SEQ ID NO: 32 - DNA, 46 bp, Chikungunya virus
  misc_feature (39)..(39): n is a, c, g, or t
tgggctgtaccgtttgtagataactgcggccaatacttntacggct

SEQ ID NO: 33 - DNA, 43 bp, Chikungunya virus
ccggcctcctgagtactgtactgctccgtggtgccagttgtag

SEQ ID NO: 34 - DNA, 40 bp, Chikungunya virus
  misc_feature (9)..(9): n is a, c, g, or t
ggtttgccngcacctgtagggatggtgaaccggcctcctg

SEQ ID NO: 35 - DNA, 43 bp, Chikungunya virus
  misc_feature (3)..(3): n is a, c, g, or t
ctnttgactagagtcttatacggtactcccaccgtgttcggga

SEQ ID NO: 36 - DNA, 51 bp, Chikungunya virus
  misc_feature (8)..(8): n is a, c, g, or t
ctgttctnatgcagcatattaggctaagcaggaaagggacggtagctcctg

SEQ ID NO: 37 - DNA, 37 bp, Chikungunya virus
ttctgttttgcatgattcggacttctccacatgtgct

SEQ ID NO: 38 - DNA, 40 bp, Chikungunya virus
  misc_feature (7)..(7): n is a, c, g, or t
agacaanttgcctcgtctaccttccgtcaggtctgttgaa

SEQ ID NO: 39 - DNA, 42 bp, Chikungunya virus
  misc_feature (6)..(6): n is a, c, g, or t
  misc_feature (9)..(9): n is a, c, g, or t
gccatnacngcttgtaagtccccgatctttccagagatgttt

SEQ ID NO: 40 - DNA, 40 bp, Chikungunya virus
ctgcgtggtgggttaccgcataccctgtggtttttccata

SEQ ID NO: 41 - DNA, 45 bp, Chikungunya virus
  misc_feature (3)..(3): n is a, c, g, or t
cangaatccgtctgcgtggtgggttaccgcataccctgtggtttt

SEQ ID NO: 42 - DNA, 42 bp, Chikungunya virus
  misc_feature (36)..(36): n is a, c, g, or t
ccggtcatttgatcacaaatggtcgccggcacgtangtgcac

SEQ ID NO: 43 - DNA, 47 bp, Chikungunya virus
tctgtagcaaggatgccggtcatttgatcacaaatggtcgccggcac

SEQ ID NO: 44 - DNA, 41 bp, Chikungunya virus
tcagccccaccaacagcttctgtgcatcctccggcgtgact

SEQ ID NO: 45 - DNA, 43 bp, Chikungunya virus
ttcagccccaccaacagcttctgtgcatcctccggcgtgactt

SEQ ID NO: 46 - DNA, 44 bp, Chikungunya virus
gttgaatactgctgagtccaaagtgggtaattccctcatctgtg

SEQ ID NO: 47 - DNA, 46 bp, Chikungunya virus
  misc_feature (7)..(7): n is a, c, g, or t
cttctgnattgactgggtatcaggcctcttgtagaccgtgtgtgtt

SEQ ID NO: 48 - DNA, 48 bp, Chikungunya virus
ctcattcgtagtgcgcattttgccttcgtaatgcaacgatgacacaat

SEQ ID NO: 49 - DNA, 38 bp, Chikungunya virus
  misc_feature (10)..(10): n is a, c, g, or t
cacaatggcngtcacaggcagtgtacaccgcctggaga

SEQ ID NO: 50 - DNA, 47 bp, Chikungunya virus
  misc_feature (3)..(3): n is a, c, g, or t
tgncaaaataggtagctgtagtgcgtacctatttaggaccgccgtac

SEQ ID NO: 51 - DNA, 40 bp, Chikungunya virus
  misc_feature (10)..(10): n is a, c, g, or t
catcatgctnctgtatcctgaccacccaacactcctgtcc

SEQ ID NO: 52 - DNA, 38 bp, Chikungunya virus
  misc_feature (1)..(1): n is a, c, g, or t
nacatgcagggtgcctaaagcaaggaaccccaccgtga

SEQ ID NO: 53 - DNA, 44 bp, Chikungunya virus
  misc_feature (36)..(36): n is a, c, g, or t
gggagaagaaccaaactatcaagaagagtgggtgangcataaga

SEQ ID NO: 54 - DNA, 39 bp, Chikungunya virus
  misc_feature (7)..(7): n is a, c, g, or t
taagtangaccttgaatgcgcgcagatacccgtgcacat

SEQ ID NO: 55 - DNA, 44 bp, Chikungunya virus
gatacccgtgcacatgaagtccgacgcttcgaagttcacccatg

SEQ ID NO: 56 - DNA, 41 bp, Chikungunya virus
cggtgcccacactgtgagcgcgtacgaacacgtaacagtga

SEQ ID NO: 57 - DNA, 44 bp, Chikungunya virus
  misc_feature (4)..(4): n is a, c, g, or t
  misc_feature (38)..(38): n is a, c, g, or t
cagnggggatgtgcatgtgtgcacgacgcagatgcatnacaccg

SEQ ID NO: 58 - DNA, 38 bp, Chikungunya virus
tacctgactacagctgtaaggtcttcaccggcgtctac

SEQ ID NO: 59 - DNA, 39 bp, Chikungunya virus
  misc_feature (4)..(4): n is a, c, g, or t
  misc_feature (10)..(10): n is a, c, g, or t
aaantgggcngatgagcaggtactgaaggctaagaacat

SEQ ID NO: 60 - DNA, 39 bp, Chikungunya virus
  misc_feature (10)..(10): n is a, c, g, or t
gagaaagctngcatctgccgcaggaaaagtcctggacag

SEQ ID NO: 61 - DNA, 38 bp, Chikungunya virus
  misc_feature (6)..(6): n is a, c, g, or t
  misc_feature (9)..(9): n is a, c, g, or t
  misc_feature (30)..(30): n is a, c, g, or t
ggcaanctnagcttcacatgccgctgtganacagtggt

SEQ ID NO: 62 - DNA, 43 bp, Chikungunya virus
  misc_feature (42)..(42): n is a, c, g, or t
aaaccacagggtatgcggtaacccaccacgcagacggattcnt

SEQ ID NO: 63 - DNA, 42 bp, Chikungunya virus
caagactaccgacacggttgacggcgaaagagtgtcattctc

SEQ ID NO: 64 - DNA, 38 bp, Chikungunya virus
  misc_feature (29)..(29): n is a, c, g, or t
gcgaaagagtgtcattctcggtgtgcacntacgtgccg

SEQ ID NO: 65 - DNA, 40 bp, Chikungunya virus
  misc_feature (40)..(40): n is a, c, g, or t
gaacacactacagaatgtactggcagcagccacgaaaagn

SEQ ID NO: 66 - DNA, 43 bp, Chikungunya virus
  misc_feature (34)..(34): n is a, c, g, or t
actacagaatgtactggcagcagccacgaaaagnaactgcaac

SEQ ID NO: 67 - DNA, 37 bp, Chikungunya virus
  misc_feature (10)..(10): n is a, c, g, or t
  misc_feature (34)..(34): n is a, c, g, or t
aagaacactnacctgctgctgtctatgggcattnaag

SEQ ID NO: 68 - DNA, 39 bp, Chikungunya virus
acccgaagcagtgcggcttcttcaatatgatgcagatga

SEQ ID NO: 69 - DNA, 39 bp, Chikungunya virus
  misc_feature (1)..(1): n is a, c, g, or t
nggtaatgtccatggccacctttgcaagctccagatcca

SEQ ID NO: 70 - DNA, 39 bp, Chikungunya virus
acccaacactcctgtcctaccggaatatgggagaagaac

SEQ ID NO: 71 - DNA, 39 bp, Chikungunya virus
cctgtcctaccggaatatgggagaagaaccaaactatca

SEQ ID NO: 72 - DNA, 42 bp, Chikungunya virus
  misc_feature (41)..(41): n is a, c, g, or t
ctgaagggctcgaggtcacgtggggcaacaacgagccgtana

SEQ ID NO: 73 - DNA, 44 bp, Chikungunya virus
gttcacccatgagaaaccggaggggtactacaactggcaccacg

SEQ ID NO: 74 - DNA, 40 bp, Chikungunya virus
gtacgaacacgtaacagtgatcccgaacacggtgggagta

SEQ ID NO: 75 - DNA, 37 bp, Chikungunya virus
  misc_feature (7)..(7): n is a, c, g, or t
accgtangaactgacaccaggagctaccgtccctttc

SEQ ID NO: 76 - DNA, 34 bp, Chikungunya virus
  misc_feature (27)..(27): n is a, c, g, or t
ggggcggcgcctactgcttctgcgacnctgaaaa

SEQ ID NO: 77 - DNA, 38 bp, Chikungunya virus
taagaacataggattatgttcaacagacctgacggaag

SEQ ID NO: 78 - DNA, 38 bp, Chikungunya virus
caggaaaagtcctggacagaaacatctctggaaagatc

SEQ ID NO: 79 - DNA, 38 bp, Chikungunya virus
tgagggctacgtcgttaagagaataacgatgagcccag

SEQ ID NO: 80 - DNA, 38 bp, Chikungunya virus; identical to SEQ ID NO: 64
  misc_feature (29)..(29): n is a, c, g, or t

SEQ ID NO: 81 - DNA, 39 bp, Chikungunya virus
gtgccggcgaccatttgtgatcaaatgaccggcatcctt

SEQ ID NO: 82 - DNA, 39 bp, Chikungunya virus
  misc_feature (8)..(8): n is a, c, g, or t
cgaaaagnaactgcaacgtcacacagatgagggaattac

SEQ ID NO: 83 - DNA, 38 bp, Chikungunya virus
  misc_feature (8)..(8): n is a, c, g, or t
gggcattnaagaagcagaaaacacacacggtctacaag

SEQ ID NO: 84 - DNA, 40 bp, Chikungunya virus
  misc_feature (3)..(3): n is a, c, g, or t
  misc_feature (9)..(9): n is a, c, g, or t
tanaatcanaacatctgcacccaagtgtaccacaaaagta

SEQ ID NO: 85 - DNA, 40 bp, Chikungunya virus
tccaacttcgagaagctcagaggacccgtcataactttgt

SEQ ID NO: 86 - RNA, 48 nt, Chikungunya virus
  misc_feature (42)..(42): n is a, c, g, or u
uuguguagaacagacuuguacgcggaauucggcgcuggcuanggccgu

SEQ ID NO: 87 - RNA, 51 nt, Chikungunya virus
  misc_feature (46)..(46): n is a, c, g, or u
  misc_feature (49)..(49): n is a, c, g, or u
ggauacaacugcaucuaugaucuucacuuccauguucauccaagungcnca

SEQ ID NO: 88 - RNA, 48 nt, Chikungunya virus
gcaaacgccucgucuacguacaacacgucgacuggucuguugcaucca

SEQ ID NO: 89 - RNA, 46 nt, Chikungunya virus
  misc_feature (4)..(4): n is a, c, g, or u
  misc_feature (6)..(7): n is a, c, g, or u
  misc_feature (10)..(10): n is a, c, g, or u
  misc_feature (46)..(46): n is a, c, g, or u
agunannuunuuuccuugguaaaggacgcggagcuuagcugaugcn

SEQ ID NO: 90 - DNA, 27 bp, Artificial
  Synthetic promoter for T7 RNA polymerase
aatttaatacgactcactatagggaga

SEQ ID NO: 91 - DNA, 24 bp, Chikungunya virus
cacccactcttcttgatagtttgg

SEQ ID NO: 92 - DNA, 26 bp, Chikungunya virus
cgtttgtagataactgcggccaatac

SEQ ID NO: 93 - DNA, 23 bp, Chikungunya virus
gagtactgtactgctccgtggtg

SEQ ID NO: 94 - DNA, 20 bp, Chikungunya virus
cacctgtagggatggtgaac

SEQ ID NO: 95 - DNA, 23 bp, Chikungunya virus
gagtcttatacggtactcccacc

SEQ ID NO: 96 - DNA, 31 bp, Chikungunya virus
gcagcatattaggctaagcaggaaagggacg

SEQ ID NO: 97 - DNA, 18 bp, Chikungunya virus
gcatgattcggacttctc

SEQ ID NO: 98 - DNA, 20 bp, Chikungunya virus
cctcgtctaccttccgtcag

SEQ ID NO: 99 - DNA, 23 bp, Chikungunya virus
gcttgtaagtccccgatctttcc

SEQ ID NO: 100 - DNA, 20 bp, Chikungunya virus
ggttaccgcataccctgtgg

SEQ ID NO: 101 - DNA, 25 bp, Chikungunya virus
tctgcgtggtgggttaccgcatacc

SEQ ID NO: 102 - DNA, 22 bp, Chikungunya virus
gatcacaaatggtcgccggcac

SEQ ID NO: 103 - DNA, 27 bp, Chikungunya virus
ggatgccggtcatttgatcacaaatgg

SEQ ID NO: 104 - DNA, 21 bp, Chikungunya virus
caacagcttctgtgcatcctc

SEQ ID NO: 105 - DNA, 23 bp, Chikungunya virus
ccaacagcttctgtgcatcctcc

SEQ ID NO: 106 - DNA, 24 bp, Chikungunya virus
gctgagtccaaagtgggtaattcc

SEQ ID NO: 107 - DNA, 26 bp, Chikungunya virus
gactgggtatcaggcctcttgtagac

SEQ ID NO: 108 - DNA, 28 bp, Chikungunya virus
gtgcgcattttgccttcgtaatgcaacg

SEQ ID NO: 109 - DNA, 18 bp, Chikungunya virus
gtcacaggcagtgtacac

SEQ ID NO: 110 - DNA, 27 bp, Chikungunya virus
ggtagctgtagtgcgtacctatttagg

SEQ ID NO: 111 - DNA, 51 bp, Artificial
  T7 promoter-primer for amplifying CHIKV nucleic acids in System 1
aatttaatacgactcactatagggagacacccactcttcttgatagtttgg

SEQ ID NO: 112 - DNA, 53 bp, Artificial
  T7 promoter-primer for amplifying CHIKV nucleic acids in System 2
aatttaatacgactcactatagggagacgtttgtagataactgcggccaatac

SEQ ID NO: 113 - DNA, 50 bp, Artificial
  T7 promoter-primer for amplifying CHIKV nucleic acids in System 3
aatttaatacgactcactatagggagagagtactgtactgctccgtggtg

SEQ ID NO: 114 - DNA, 47 bp, Artificial
  T7 promoter-primer for amplifying CHIKV nucleic acids in System 3
aatttaatacgactcactatagggagacacctgtagggatggtgaac

SEQ ID NO: 115 - DNA, 50 bp, Artificial
  T7 promoter-primer for amplifying CHIKV nucleic acids in System 4
aatttaatacgactcactatagggagagagtcttatacggtactcccacc

SEQ ID NO: 116 - DNA, 58 bp, Artificial
  T7 promoter-primer for amplifying CHIKV nucleic acids in System 5
aatttaatacgactcactatagggagagcagcatattaggctaagcaggaaagggacg

SEQ ID NO: 117 - DNA, 45 bp, Artificial
  T7 promoter-primer for amplifying CHIKV nucleic acids in System 6
aatttaatacgactcactatagggagagcatgattcggacttctc

SEQ ID NO: 118 - DNA, 47 bp, Artificial
  T7 promoter-primer for amplifying CHIKV nucleic acids in System 7
aatttaatacgactcactatagggagacctcgtctaccttccgtcag

SEQ ID NO: 119 - DNA, 50 bp, Artificial
  T7 promoter-primer for amplifying CHIKV nucleic acids in System 8
aatttaatacgactcactatagggagagcttgtaagtccccgatctttcc

SEQ ID NO: 120 - DNA, 47 bp, Artificial
  T7 promoter-primer for amplifying CHIKV nucleic acids in System 9
aatttaatacgactcactatagggagaggttaccgcataccctgtgg

SEQ ID NO: 121 - DNA, 52 bp, Artificial
  T7 promoter-primer for amplifying CHIKV nucleic acids in System 9
aatttaatacgactcactatagggagatctgcgtggtgggttaccgcatacc

SEQ ID NO: 122 - DNA, 49 bp, Artificial
  T7 promoter-primer for amplifying CHIKV nucleic acids in System 10
aatttaatacgactcactatagggagagatcacaaatggtcgccggcac

SEQ ID NO: 123 - DNA, 54 bp, Artificial
  T7 promoter-primer for amplifying CHIKV nucleic acids in System 10
aatttaatacgactcactatagggagaggatgccggtcatttgatcacaaatgg

SEQ ID NO: 124 - DNA, 48 bp, Artificial
  T7 promoter-primer for amplifying CHIKV nucleic acids in System 11
aatttaatacgactcactatagggagacaacagcttctgtgcatcctc

SEQ ID NO: 125 - DNA, 50 bp, Artificial
  T7 promoter-primer for amplifying CHIKV nucleic acids in System 11
aatttaatacgactcactatagggagaccaacagcttctgtgcatcctcc

SEQ ID NO: 126 - DNA, 51 bp, Artificial
  T7 promoter-primer for amplifying CHIKV nucleic acids in System 12
aatttaatacgactcactatagggagagctgagtccaaagtgggtaattcc

SEQ ID NO: 127 - DNA, 53 bp, Artificial
  T7 promoter-primer for amplifying CHIKV nucleic acids in System 13
aatttaatacgactcactatagggagagactgggtatcaggcctcttgtagac

SEQ ID NO: 128 - DNA, 55 bp, Artificial
  T7 promoter-primer for amplifying CHIKV nucleic acids in System 14
aatttaatacgactcactatagggagagtgcgcattttgccttcgtaatgcaacg

SEQ ID NO: 129 - DNA, 45 bp, Artificial
  T7 promoter-primer for amplifying CHIKV nucleic acids in System 14
aatttaatacgactcactatagggagagtcacaggcagtgtacac

SEQ ID NO: 130 - DNA, 54 bp, Artificial
  T7 promoter-primer for amplifying CHIKV nucleic acids in System 15
aatttaatacgactcactatagggagaggtagctgtagtgcgtacctatttagg

SEQ ID NO: 131 - DNA, 20 bp, Chikungunya virus
ctgtatcctgaccacccaac

SEQ ID NO: 132 - DNA, 18 bp, Chikungunya virus
gtgcctaaagcaaggaac

SEQ ID NO: 133 - DNA, 24 bp, Chikungunya virus
ccaaactatcaagaagagtgggtg

SEQ ID NO: 134 - DNA, 19 bp, Chikungunya virus
cttgaatgcgcgcagatac

SEQ ID NO: 135 - DNA, 24 bp, Chikungunya virus
cacatgaagtccgacgcttcgaag

SEQ ID NO: 136 - DNA, 21 bp, Chikungunya virus
actgtgagcgcgtacgaacac

SEQ ID NO: 137 - DNA, 24 bp, Chikungunya virus
gtgcatgtgtgcacgacgcagatg

SEQ ID NO: 138 - DNA, 18 bp, Chikungunya virus
cagctgtaaggtcttcac

SEQ ID NO: 139 - DNA, 19 bp, Chikungunya virus
gatgagcaggtactgaagg

SEQ ID NO: 140 - DNA, 19 bp, Chikungunya virus
gcatctgccgcaggaaaag

SEQ ID NO: 141 - DNA, 18 bp, Chikungunya virus
gcttcacatgccgctgtg

SEQ ID NO: 142 - DNA, 23 bp, Chikungunya virus
gtatgcggtaacccaccacgcag

SEQ ID NO: 143 - DNA, 22 bp, Chikungunya virus
gacacggttgacggcgaaagag

SEQ ID NO: 144 - DNA, 18 bp, Chikungunya virus
gtcattctcggtgtgcac

SEQ ID NO: 145 - DNA, 20 bp, Chikungunya virus
cagaatgtactggcagcagc

SEQ ID NO: 146 - DNA, 23 bp, Chikungunya virus
gtactggcagcagccacgaaaag

SEQ ID NO: 147 - DNA, 17 bp, Chikungunya virus
acctgctgctgtctatg

SEQ ID NO: 148 - DNA, 19 bp, Chikungunya virus
gtgcggcttcttcaatatg

SEQ ID NO: 149 - DNA, 19 bp, Chikungunya virus
catggccacctttgcaagc

SEQ ID NO: 150 - RNA, 19 nt, Chikungunya virus
ccuguccuaccggaauaug

SEQ ID NO: 151 - RNA, 19 nt, Chikungunya virus
cggaauaugggagaagaac

SEQ ID NO: 152 - RNA, 22 nt, Chikungunya virus
cgaggucacguggggcaacaac

SEQ ID NO: 153 - RNA, 24 nt, Chikungunya virus
gagaaaccggagggguacuacaac

SEQ ID NO: 154 - RNA, 19 nt, Chikungunya virus
guaacagugaucccgaaca

SEQ ID NO: 155 - DNA, 17 bp, Chikungunya virus
ctgacaccaggagctac

SEQ ID NO: 156 - RNA, 16 nt, Chikungunya virus
cuacugcuucugcgac

SEQ ID NO: 157 - RNA, 18 nt, Chikungunya virus
ggauuauguucaacagac

SEQ ID NO: 158 - RNA, 18 nt, Chikungunya virus
ccuggacagaaacaucuc

SEQ ID NO: 159 - RNA, 18 nt, Chikungunya virus
gucguuaagagaauaacg

SEQ ID NO: 160 - RNA, 18 nt, Chikungunya virus
gucauucucggugugcac

SEQ ID NO: 161 - RNA, 19 nt, Chikungunya virus
ccauuugugaucaaaugac

SEQ ID NO: 162 - RNA, 19 nt, Chikungunya virus
cugcaacgucacacagaug

SEQ ID NO: 163 - RNA, 18 nt, Chikungunya virus
gaagcagaaaacacacac

SEQ ID NO: 164 - RNA, 20 nt, Chikungunya virus
acaucugcacccaaguguac

SEQ ID NO: 165 - RNA, 20 nt, Chikungunya virus
agaagcucagaggacccguc

SEQ ID NO: 166 - RNA, 28 nt, Chikungunya virus
cagacuuguacgcggaauucggcgcugg

SEQ ID NO: 167 - RNA, 51 nt, Chikungunya virus; identical to SEQ ID NO: 87
  misc_feature (46)..(46): n is a, c, g, or u
  misc_feature (49)..(49): n is a, c, g, or u

SEQ ID NO: 168 - RNA, 48 nt, Chikungunya virus; identical to SEQ ID NO: 88

SEQ ID NO: 169 - RNA, 46 nt, Chikungunya virus; identical to SEQ ID NO: 89
  misc_feature (4)..(4): n is a, c, g, or u
  misc_feature (6)..(7): n is a, c, g, or u
  misc_feature (10)..(10): n is a, c, g, or u
  misc_feature (46)..(46): n is a, c, g, or u

SEQ ID NO: 170 - DNA, 19 bp, Chikungunya virus
cttcaatatgatgcagatg

SEQ ID NO: 171 - DNA, 19 bp, Chikungunya virus
gatgcagatgaaagtcaac

SEQ ID NO: 172 - DNA, 19 bp, Chikungunya virus
cagtgcggcttcttcaata

SEQ ID NO: 173 - DNA, 19 bp, Chikungunya virus
ggcttcttcaatatgatgc

SEQ ID NO: 174 - DNA, 20 bp, Chikungunya virus
acatctgcacccaagtgtac

SEQ ID NO: 175 - DNA, 17 bp, Chikungunya virus
tgcacccaagtgtacca

SEQ ID NO: 176 - DNA, 17 bp, Chikungunya virus
aacatctgcacccaagt

SEQ ID NO: 177 - DNA, 29 bp, Chikungunya virus
agtgcgcattttgccttcgtaatgcaacg

SEQ ID NO: 178 - DNA, 18 bp, Chikungunya virus
ccgcctggagatactttt

SEQ ID NO: 179 - DNA, 19 bp, Chikungunya virus
accgcctggagatactttt

SEQ ID NO: 180 - DNA, 21 bp, Chikungunya virus
agaccgcctggagatactttt

SEQ ID NO: 181 - DNA, 23 bp, Chikungunya virus
ggagaccgcctggagatactttt

SEQ ID NO: 182 - DNA, 45 bp, Artificial
  T7 promoter-primer for amplifying CHIKV nucleic acids in System 14
aatttaatacgactcactatagggagaccgcctggagatactttt

SEQ ID NO: 183 - RNA, 17 nt, Chikungunya virus
ccugugacygccauugu

SEQ ID NO: 184 - RNA, 17 nt, Chikungunya virus
ccugugacugccauugu

SEQ ID NO: 185 - RNA, 17 nt, Chikungunya virus
ccugugaccgccauugu

SEQ ID NO: 186 - DNA, 87 bp, Chikungunya virus
  misc_feature (50)..(50): n is a, c, g, or t
  misc_feature (56)..(56): n is a, c, g, or t
acccgaagcagtgcggcttcttcaatatgatgcagatgaaagtcaactanaatcanaacatctgcacccaagtgtaccacaaaagta

SEQ ID NO: 187 - DNA, 47 bp, Chikungunya virus
acccgaagcagtgcggcttcttcaatatgatgcagatgaaagtcaac

SEQ ID NO: 188 - RNA, 28 nt, Chikungunya virus
cagacuuguacgcggaauucggcgcugg

SEQ ID NO: 189 - RNA, 31 nt, Chikungunya virus
gcaucuaugaucuucacuuccauguucaucc

SEQ ID NO: 190 - RNA, 28 nt, Chikungunya virus
cgucuacguacaacacgucgacuggucu

SEQ ID NO: 191 - RNA, 26 nt, Chikungunya virus
uuuccuugguaaaggacgcggagcuu